European Patent Specification EP 4 013 413 B1, published January 29, 2025. Title: Targeting WNK1 in blood cancers. Applicant: University of Copenhagen. The sequence listing filed with the application follows.

SEQUENCE LISTING (7 sequences)

SEQ ID NO: 1 - DNA, 20 bp, Lentivirus
  misc_RNA (1)..(20)
tggtctggcaactctaaagc

SEQ ID NO: 2 - DNA, 20 bp, Lentivirus
  misc_RNA (1)..(20)
tctggacaccgaaaccactg

SEQ ID NO: 3 - DNA, 20 bp, Lentivirus
  misc_RNA (1)..(20)
attctcttggttctaggtcc

SEQ ID NO: 4 - DNA, 20 bp, Lentivirus
  misc_RNA (1)..(20)
gacgtctaatttctggccgt

SEQ ID NO: 5 - DNA, 20 bp, Lentivirus
  misc_RNA (1)..(20)
gccgtgggaatgtctaacga

SEQ ID NO: 6 - DNA, 20 bp, Lentivirus
  misc_RNA (1)..(20)
cgaatgggtggataccgtca

SEQ ID NO: 7 - DNA, 20 bp, Lentivirus
  misc_RNA (1)..(20)
cccgcatgacaccgtcactt